European Patent Specification EP 4 055 055 B1, published November 22, 2023. Title: BISPECIFIC ANTIBODIES AGAINST CEACAM5 AND CD47. Applicant: LAMKAP BIO BETA AG BUATOIS, VANESSA HOSE, DIRK SECKINGER, ANJA. The sequence listing filed with the application follows.

SEQUENCE LISTING (50 sequences)

SEQ ID NO: 1 - protein, 5 aa, Artificial Sequence
  Common heavy chain CDRH1
SYAMS

SEQ ID NO: 2 - protein, 17 aa, Artificial Sequence
  Common heavy chain CDRH2
AISGSGGSTYYADSVKG

SEQ ID NO: 3 - protein, 7 aa, Artificial Sequence
  Common heavy chain CDRH3
SYGAFDY

SEQ ID NO: 4 - protein, 116 aa, Artificial Sequence
  Common heavy chain VH
EVQLLESGGGLVQPGGSLRLSCAASGFTFSSYAMSWVRQAPGKGLEWVSAISGSGGSTYYADSVKGRFTISRDNSKNTLYLQMNSLRAEDTAVYYCAKSYGAFDYWGQGTLVTVSS

SEQ ID NO: 5 - protein, 229 aa, Artificial Sequence
  Common heavy chain (VH-CH1)
EVQLLESGGGLVQPGGSLRLSCAASGFTFSSYAMSWVRQAPGKGLEWVSAISGSGGSTYYADSVKGRFTISRDNSKNTLYLQMNSLRAEDTAVYYCAKSYGAFDYWGQGTLVTVSSASTKGPSVFPLAPSSKSTSGGTAALGCLVKDYFPEPVTVSWNSGALTSGVHTFPAVLQSSGLYSLSSVVTVPSSSLGTQTYICNVNHKPSNTKVDKRVEPKSCDKTHTCPPCP

SEQ ID NO: 6 - protein, 445 aa, Artificial Sequence
  common heavy chain (VH-CH1-CH2-CH3)
EVQLLESGGGLVQPGGSLRLSCAASGFTFSSYAMSWVRQAPGKGLEWVSAISGSGGSTYYADSVKGRFTISRDNSKNTLYLQMNSLRAEDTAVYYCAKSYGAFDYWGQGTLVTVSSASTKGPSVFPLAPSSKSTSGGTAALGCLVKDYFPEPVTVSWNSGALTSGVHTFPAVLQSSGLYSLSSVVTVPSSSLGTQTYICNVNHKPSNTKVDKRVEPKSCDKTHTCPPCPAPELLGGPSVFLFPPKPKDTLMISRTPEVTCVVVDVSHEDPEVKFNWYVDGVEVHNAKTKPREEQYNSTYRVVSVLTVLHQDWLNGKEYKCKVSNKALPAPIEKTISKAKGQPREPQVYTLPPSREEMTKNQVSLTCLVKGFYPSDIAVEWESNGQPENNYKTTPPVLDSDGSFFLYSKLTVDKSRWQQGNVFSCSVMHEALHNHYTQKSLSLSPG

SEQ ID NO: 7 - protein, 11 aa, Artificial Sequence
  CD47 binding part CDRL1
RASQSISSYLN

SEQ ID NO: 8 - protein, 7 aa, Artificial Sequence
  CD47 binding part CDRL2
AASSLQS

SEQ ID NO: 9 - protein, 10 aa, Artificial Sequence
  CD47 binding part CDRL3
QQMHPRAPKT

SEQ ID NO: 10 - protein, 108 aa, Artificial Sequence
  CD47 binding part VK
DIQMTQSPSSLSASVGDRVTITCRASQSISSYLNWYQQKPGKAPKLLIYAASSLQSGVPSRFSGSGSGTDFTLTISSLQPEDFATYYCQQMHPRAPKTFGQGTKVEIK

SEQ ID NO: 11 - protein, 215 aa, Artificial Sequence
  CD47 binding part light chain (VKCK; K2)
DIQMTQSPSSLSASVGDRVTITCRASQSISSYLNWYQQKPGKAPKLLIYAASSLQSGVPSRFSGSGSGTDFTLTISSLQPEDFATYYCQQMHPRAPKTFGQGTKVEIKRTVAAPSVFIFPPSDEQLKSGTASVVCLLNNFYPREAKVQWKVDNALQSGNSQESVTEQDSKDSTYSLSSTLTLSKADYEKHKVYACEVTHQGLSSPVTKSFNRGEC

SEQ ID NO: 12 - DNA, 648 bp, Artificial Sequence
  CD47 binding part light chain (VKCK; nucleic acid); (K2)
gacatccagatgacccagtctccatcctccctgtctgcatctgtaggagacagagtcaccatcacttgccgggcaagtcagagcattagcagctatttaaattggtatcagcagaaaccagggaaagcccctaagctcctgatctatgctgcatccagtttgcaaagtggggtcccatcaaggttcagtggcagtggatctgggacagatttcactctcaccatcagcagtctgcaacctgaagattttgcaacttactactgtcagcagatgcacccgcgcgccccgaagaccttcggccaagggaccaaggtggaaatcaaacgtacggtggctgcaccatctgtcttcatcttcccgccatctgatgagcagttgaaatctggaactgcctctgttgtgtgcctgctgaataacttctatcccagagaggccaaagtacagtggaaggtggataacgccctccaatcgggtaactcccaggagagtgtcacagagcaggacagcaaggacagcacctacagcctcagcagcaccctgacgctgagcaaagcagactacgagaaacacaaagtctacgcctgcgaagtcacccatcagggcctgagctcgcccgtcacaaagagcttcaacaggggagagtgttaa

SEQ ID NO: 13 - protein, 107 aa, Artificial Sequence [sequence omitted]

SEQ ID NO: 14 - protein, 13 aa, Artificial Sequence
  CEACAM5 binding part AC82 CDRL1;
SGSSSNIGYGLVS

SEQ ID NO: 15 - protein, 7 aa, Artificial Sequence
  CEACAM5 binding part AC82 CDRL2
GINKRPS

SEQ ID NO: 16 - protein, 10 aa, Artificial Sequence
  CEACAM5 binding part AC82 CDRL3
GTWDFSYRVD

SEQ ID NO: 17 - protein, 13 aa, Artificial Sequence
  CEACAM5 binding part AC84 CDRL1
SGSSSNIGIGLVS

SEQ ID NO: 18 - protein, 7 aa, Artificial Sequence
  CEACAM5 binding part AC84 CDRL2
NVNTRPS

SEQ ID NO: 19 - protein, 10 aa, Artificial Sequence
  CEACAM5 binding part AC84 CDRL3
GTWDFSYRVD

SEQ ID NO: 20 - protein, 13 aa, Artificial Sequence
  CEACAM5 binding part AC91 CDRL1
SGSSSNIGIGLVS

SEQ ID NO: 21 - protein, 7 aa, Artificial Sequence
  CEACAM5 binding part AC91 CDRL2
TVNNRPS

SEQ ID NO: 22 - protein, 10 aa, Artificial Sequence
  CEACAM5 binding part AC91 CDRL3
GTFDFSYGIV

SEQ ID NO: 23 - protein, 13 aa, Artificial Sequence
  CEACAM5 binding part AC100 CDRL1
SGSSSNIGYGLVS

SEQ ID NO: 24 - protein, 7 aa, Artificial Sequence
  CEACAM5 binding part AC100 CDRL2
NGNIRPS

SEQ ID NO: 25 - protein, 10 aa, Artificial Sequence
  CEACAM5 binding part AC100 CDRL3
GTWDFSYRVD

SEQ ID NO: 26 - protein, 13 aa, Artificial Sequence
  CEACAM5 binding part AC117 CDRL1
SGSSSNIGIGLVS

SEQ ID NO: 27 - protein, 7 aa, Artificial Sequence
  CEACAM5 binding part AC117 CDRL2
NGNVRPS

SEQ ID NO: 28 - protein, 10 aa, Artificial Sequence
  CEACAM5 binding part AC117 CDRL3
GTWDFSYRVD

SEQ ID NO: 29 - protein, 13 aa, Artificial Sequence
  CEACAM5 binding part AC22 CDRL1
SGSSSNIANGIVS

SEQ ID NO: 30 - protein, 7 aa, Artificial Sequence
  CEACAM5 binding part AC22 CDRL2
FDNLRPS

SEQ ID NO: 31 - protein, 10 aa, Artificial Sequence
  CEACAM5 binding part AC22 CDRL3
GTWDFSYGIV

SEQ ID NO: 32 - protein, 109 aa, Artificial Sequence
  CEACAM5 binding part AC82 VL
QSVLTQPPSVSAAPGQKVTISCSGSSSNIGYGLVSWYQQLPGTAPKLLIYGINKRPSGIPDRFSGSKSGTSATLGITGLQTGDEADYYCGTWDFSYRVDFGGGTKLTVL

SEQ ID NO: 33 - protein, 109 aa, Artificial Sequence
  CEACAM5 binding part AC84 VL
QSVLTQPPSVSAAPGQKVTISCSGSSSNIGIGLVSWYQQLPGTAPKLLIYNVNTRPSGIPDRFSGSKSGTSATLGITGLQTGDEADYYCGTWDFSYRVDFGGGTKLTVL

SEQ ID NO: 34 - protein, 109 aa, Artificial Sequence
  CEACAM5 binding part AC91 VL
QSVLTQPPSVSAAPGQKVTISCSGSSSNIGIGLVSWYQQLPGTAPKLLIYTVNNRPSGIPDRFSGSKSGTSATLGITGLQTGDEADYYCGTFDFSYGIVFGGGTKLTVL

SEQ ID NO: 35 - protein, 109 aa, Artificial Sequence
  CEACAM5 binding part AC100 VL
QSVLTQPPSVSAAPGQKVTISCSGSSSNIGYGLVSWYQQLPGTAPKLLIYNGNIRPSGIPDRFSGSKSGTSATLGITGLQTGDEADYYCGTWDFSYRVDFGGGTKLTVL

SEQ ID NO: 36 - protein, 109 aa, Artificial Sequence
  CEACAM5 binding part AC117 VL
QSVLTQPPSVSAAPGQKVTISCSGSSSNIGIGLVSWYQQLPGTAPKLLIYNGNVRPSGIPDRFSGSKSGTSATLGITGLQTGDEADYYCGTWDFSYRVDFGGGTKLTVL

SEQ ID NO: 37 - protein, 215 aa, Artificial Sequence
  CEACAM5 binding part AC82 VLCL
QSVLTQPPSVSAAPGQKVTISCSGSSSNIGYGLVSWYQQLPGTAPKLLIYGINKRPSGIPDRFSGSKSGTSATLGITGLQTGDEADYYCGTWDFSYRVDFGGGTKLTVLGQPKAAPSVTLFPPSSEELQANKATLVCLISDFYPGAVTVAWKADSSPVKAGVETTTPSKQSNNKYAASSYLSLTPEQWKSHRSYSCQVTHEGSTVEKTVAPTECS

SEQ ID NO: 38 - protein, 215 aa, Artificial Sequence
  CEACAM5 binding part AC84 VLCL
QSVLTQPPSVSAAPGQKVTISCSGSSSNIGIGLVSWYQQLPGTAPKLLIYNVNTRPSGIPDRFSGSKSGTSATLGITGLQTGDEADYYCGTWDFSYRVDFGGGTKLTVLGQPKAAPSVTLFPPSSEELQANKATLVCLISDFYPGAVTVAWKADSSPVKAGVETTTPSKQSNNKYAASSYLSLTPEQWKSHRSYSCQVTHEGSTVEKTVAPTECS

SEQ ID NO: 39 - protein, 215 aa, Artificial Sequence
  CEACAM5 binding part AC91 VLCL
QSVLTQPPSVSAAPGQKVTISCSGSSSNIGIGLVSWYQQLPGTAPKLLIYTVNNRPSGIPDRFSGSKSGTSATLGITGLQTGDEADYYCGTFDFSYGIVFGGGTKLTVLGQPKAAPSVTLFPPSSEELQANKATLVCLISDFYPGAVTVAWKADSSPVKAGVETTTPSKQSNNKYAASSYLSLTPEQWKSHRSYSCQVTHEGSTVEKTVAPTECS

SEQ ID NO: 40 - protein, 215 aa, Artificial Sequence
  CEACAM5 binding part AC100 VLCL
QSVLTQPPSVSAAPGQKVTISCSGSSSNIGYGLVSWYQQLPGTAPKLLIYNGNIRPSGIPDRFSGSKSGTSATLGITGLQTGDEADYYCGTWDFSYRVDFGGGTKLTVLGQPKAAPSVTLFPPSSEELQANKATLVCLISDFYPGAVTVAWKADSSPVKAGVETTTPSKQSNNKYAASSYLSLTPEQWKSHRSYSCQVTHEGSTVEKTVAPTECS

SEQ ID NO: 41 - protein, 215 aa, Artificial Sequence
  CEACAM5 binding part AC117 VLCL
QSVLTQPPSVSAAPGQKVTISCSGSSSNIGIGLVSWYQQLPGTAPKLLIYNGNVRPSGIPDRFSGSKSGTSATLGITGLQTGDEADYYCGTWDFSYRVDFGGGTKLTVLGQPKAAPSVTLFPPSSEELQANKATLVCLISDFYPGAVTVAWKADSSPVKAGVETTTPSKQSNNKYAASSYLSLTPEQWKSHRSYSCQVTHEGSTVEKTVAPTECS

SEQ ID NO: 42 - protein, 215 aa, Artificial Sequence
  CEACAM5 binding part AC22 VLCL
QSVLTQPPSVSAAPGQKVTISCSGSSSNIANGIVSWYQQLPGTAPKLLIYFDNLRPSGIPDRFSGSKSGTSATLGITGLQTGDEADYYCGTWDFSYGIVFGGGTKLTVLGQPKAAPSVTLFPPSSEELQANKATLVCLISDFYPGAVTVAWKADSSPVKAGVETTTPSKQSNNKYAASSYLSLTPEQWKSHRSYSCQVTHEGSTVEKTVAPTECS

SEQ ID NO: 43 - protein, 106 aa, Artificial Sequence
  VK_SM3E
ENVLTQSPSSMSVSVGDRVNIACSASSSVPYMHWLQQKPGKSPKLLIYLTSNLASGVPSRFSGSGSGTDYSLTISSVQPEDAATYYCQQRSSYPLTFGGGTKLEIK

SEQ ID NO: 44 - protein, 120 aa, Artificial Sequence
  VH_SM3E
QVKLEQSGAEVVKPGASVKLSCKASGFNIKDSYMHWLRQGPGQRLEWIGWIDPENGDTEYAPKFQGKATFTTDTSANTAYLGLSSLRPEDTAVYYCNEGTPTGPYYFDYWGQGTLVTVSS

SEQ ID NO: 45 - DNA, 24 bp, Artificial Sequence
  Primer
gtctgaagcattatgtgttgaagc

SEQ ID NO: 46 - DNA, 23 bp, Artificial Sequence
  Primer
gtgagtacattcattgtactgtg

SEQ ID NO: 47 - DNA, 24 bp, Artificial Sequence
  Primer
ttgtgtgactcttaactctcagag

SEQ ID NO: 48 - DNA, 25 bp, Artificial Sequence
  Primer
gaggccacttgtgtagcgccaagtg

SEQ ID NO: 49 - DNA, 21 bp, Artificial Sequence
  Primer
gtgagtccatggctgtcactg

SEQ ID NO: 50 - DNA, 20 bp, Artificial Sequence
  Primer
cctgacttggctattctcag